European Patent Specification EP 3 697 401 B1, published December 3, 2025. Title: DOMINANT NEGATIVE SARM1 MOLECULES AS A THERAPEUTIC STRATEGY FOR NEURODEGENERATIVE DISEASES OR DISORDERS. Applicant: Washington University DiAntonio, Aaron Milbrandt, Jeffrey Summers, Daniel Geisler, Stefanie Mao, Xianrong. The sequence listing filed with the application follows.

SEQUENCE LISTING (15 sequences)

SEQ ID NO: 1 - protein, 724 aa, Artificial Sequence
  SYNTHESIZED
MVLTLLLSAYKLCRFFAMSGPRPGAERLAVPGPDGGGGTGPWWAAGGRGPREVSPGAGTEVQDALERALPELQQALSALKQAGGARAVGAGLAEVFQLVEEAWLLPAVGREVAQGLCDAIRLDGGLDLLLRLLQAPELETRVQAARLLEQILVAENRDRVARIGLGVILNLAKEREPVELARSVAGILEHMFKHSEETCQRLVAAGGLDAVLYWCRRTDPALLRHCALALGNCALHGGQAVQRRMVEKRAAEWLFPLAFSKEDELLRLHACLAVAVLATNKEVEREVERSGTLALVEPLVASLDPGRFARCLVDASDTSQGRGPDDLQRLVPLLDSNRLEAQCIGAFYLCAEAAIKSLQGKTKVFSDIGAIQSLKRLVSYSTNGTKSALAKRALRLLGEEVPRPILPSVPSWKEAEVQTWLQQIGFSKYCESFREQQVDGDLLLRLTEEELQTDLGMKSGITRKRFFRELTELKTFANYSTCDRSNLADWLGSLDPRFRQYTYGLVSCGLDRSLLHRVSEQQLLEDCGIHLGVHRARILTAAREMLHSPLPCTGGKPSGDTPDVFISYRRNSGSQLASLLKVHLQLHGFSVFIDVEKLEAGKFEDKLIQSVMGARNFVLVLSPGALDKCMQDHDCKDWVHKEIVTALSCGKNIVPIIDGFEWPEPQVLPEDMQAVLTFNGIKWSHEYQEATIEKIIRFLQGRSSRDSSAGSDTSLEGAAPMGPT

SEQ ID NO: 2 - protein, 724 aa, Artificial Sequence
  SYNTHESIZED
MVLTLLLSAYKLCRFFAMSGPRPGAERLAVPGPDGGGGTGPWWAAGGRGPREVSPGAGTEVQDALERALPELQQALSALKQAGGARAVGAGLAEVFQLVEEAWLLPAVGREVAQGLCDAIRLDGGLDLLLRLLQAPELETRVQAARLLEQILVAENRDRVARIGLGVILNLAKEREPVELARSVAGILEHMYKHSEETCQRLVAAGGLDAVLYWCRRTDPALLRHCALALGNCALHGGQAVQRRMVEKRAAEWLFPLAFSKEDELLRLHACLAVAVLATNKEVEREVERSGTLALVEPLVASLDPGRFARCLVDASDTSQGRGPDDLQRLVPLLDSNRLEAQCIGAFYLCAEAAIKSLQGKTKVFSDIGAIQSLKRLVSYSTNGTKSALAKRALRLLGEEVPRPILPSVPSWKEAEVQTWLQQIGFSKYCESFREQQVDGDLLLRLTEEELQTDLGMKSGITRKRFFRELTELKTFANYSTCDRSNLADWLGSLDPRFRQYTYGLVSCGLDRSLLHRVSEQQLLEDCGIHLGVHRARILTAAREMLHSPLPCTGGKPSGDTPDVFISYRRNSGSQLASLLKVHLQLHGFSVFIDVEKLEAGKFEDKLIQSVMGARNFVLVLSPGALDKCMQDHDCKDWVHKEIVTALSCGKNIVPIIDGFEWPEPQVLPEDMQAVLTFNGIKWSHEYQEATIEKIIRFLQGRSSRDSSAGSDTSLEGAAPMGPT

SEQ ID NO: 3 - protein, 724 aa, Artificial Sequence
  SYNTHESIZED
MVLTLLLSAYKLCRFFAMSGPRPGAERLAVPGPDGGGGTGPWWAAGGRGPREVSPGAGTEVQDALERALPELQQALSALKQAGGARAVGAGLAEVFQLVEEAWLLPAVGREVAQGLCDAIRLDGGLDLLLRLLQAPELETRVQAARLLEQILVAENRDRVARIGLGVILNLAKEREPVELARSVAGILEHMFRHSEETCQRLVAAGGLDAVLYWCRRTDPALLRHCALALGNCALHGGQAVQRRMVEKRAAEWLFPLAFSKEDELLRLHACLAVAVLATNKEVEREVERSGTLALVEPLVASLDPGRFARCLVDASDTSQGRGPDDLQRLVPLLDSNRLEAQCIGAFYLCAEAAIKSLQGKTKVFSDIGAIQSLKRLVSYSTNGTKSALAKRALRLLGEEVPRPILPSVPSWKEAEVQTWLQQIGFSKYCESFREQQVDGDLLLRLTEEELQTDLGMKSGITRKRFFRELTELKTFANYSTCDRSNLADWLGSLDPRFRQYTYGLVSCGLDRSLLHRVSEQQLLEDCGIHLGVHRARILTAAREMLHSPLPCTGGKPSGDTPDVFISYRRNSGSQLASLLKVHLQLHGFSVFIDVEKLEAGKFEDKLIQSVMGARNFVLVLSPGALDKCMQDHDCKDWVHKEIVTALSCGKNIVPIIDGFEWPEPQVLPEDMQAVLTFNGIKWSHEYQEATIEKIIRFLQGRSSRDSSAGSDTSLEGAAPMGPT

SEQ ID NO: 4 - protein, 724 aa, Artificial Sequence
  SYNTHESIZED
MVLTLLLSAYKLCRFFAMSGPRPGAERLAVPGPDGGGGTGPWWAAGGRGPREVSPGAGTEVQDALERALPELQQALSALKQAGGARAVGAGLAEVFQLVEEAWLLPAVGREVAQGLCDAIRLDGGLDLLLRLLQAPELETRVQAARLLEQILVAENRDRVARIGLGVILNLAKEREPVELARSVAGILEHMFAHSEETCQRLVAAGGLDAVLYWCRRTDPALLRHCALALGNCALHGGQAVQRRMVEKRAAEWLFPLAFSKEDELLRLHACLAVAVLATNKEVEREVERSGTLALVEPLVASLDPGRFARCLVDASDTSQGRGPDDLQRLVPLLDSNRLEAQCIGAFYLCAEAAIKSLQGKTKVFSDIGAIQSLKRLVSYSTNGTKSALAKRALRLLGEEVPRPILPSVPSWKEAEVQTWLQQIGFSKYCESFREQQVDGDLLLRLTEEELQTDLGMKSGITRKRFFRELTELKTFANYSTCDRSNLADWLGSLDPRFRQYTYGLVSCGLDRSLLHRVSEQQLLEDCGIHLGVHRARILTAAREMLHSPLPCTGGKPSGDTPDVFISYRRNSGSQLASLLKVHLQLHGFSVFIDVEKLEAGKFEDKLIQSVMGARNFVLVLSPGALDKCMQDHDCKDWVHKEIVTALSCGKNIVPIIDGFEWPEPQVLPEDMQAVLTFNGIKWSHEYQEATIEKIIRFLQGRSSRDSSAGSDTSLEGAAPMGPT

SEQ ID NO: 5 - protein, 724 aa, Artificial Sequence
  SYNTHESIZED
MVLTLLLSAYKLCRFFAMSGPRPGAERLAVPGPDGGGGTGPWWAAGGRGPREVSPGAGTEVQDALERALPELQQALSALKQAGGARAVGAGLAEVFQLVEEAWLLPAVGREVAQGLCDAIRLDGGLDLLLRLLQAPELETRVQAARLLEQILVAENRDRVARIGLGVILNLAKEREPVELARSVAGILEHMFQHSEETCQRLVAAGGLDAVLYWCRRTDPALLRHCALALGNCALHGGQAVQRRMVEKRAAEWLFPLAFSKEDELLRLHACLAVAVLATNKEVEREVERSGTLALVEPLVASLDPGRFARCLVDASDTSQGRGPDDLQRLVPLLDSNRLEAQCIGAFYLCAEAAIKSLQGKTKVFSDIGAIQSLKRLVSYSTNGTKSALAKRALRLLGEEVPRPILPSVPSWKEAEVQTWLQQIGFSKYCESFREQQVDGDLLLRLTEEELQTDLGMKSGITRKRFFRELTELKTFANYSTCDRSNLADWLGSLDPRFRQYTYGLVSCGLDRSLLHRVSEQQLLEDCGIHLGVHRARILTAAREMLHSPLPCTGGKPSGDTPDVFISYRRNSGSQLASLLKVHLQLHGFSVFIDVEKLEAGKFEDKLIQSVMGARNFVLVLSPGALDKCMQDHDCKDWVHKEIVTALSCGKNIVPIIDGFEWPEPQVLPEDMQAVLTFNGIKWSHEYQEATIEKIIRFLQGRSSRDSSAGSDTSLEGAAPMGPT

SEQ ID NO: 6 - protein, 724 aa, Artificial Sequence
  SYNTHESIZED
MVLTLLLSAYKLCRFFAMSGPRPGAERLAVPGPDGGGGTGPWWAAGGRGPREVSPGAGTEVQDALERALPELQQALSALKQAGGARAVGAGLAEVFQLVEEAWLLPAVGREVAQGLCDAIRLDGGLDLLLRLLQAPELETRVQAARLLEQILVAENRDRVARIGLGVILNLAKEREPVELARSVAGILEHMFEHSEETCQRLVAAGGLDAVLYWCRRTDPALLRHCALALGNCALHGGQAVQRRMVEKRAAEWLFPLAFSKEDELLRLHACLAVAVLATNKEVEREVERSGTLALVEPLVASLDPGRFARCLVDASDTSQGRGPDDLQRLVPLLDSNRLEAQCIGAFYLCAEAAIKSLQGKTKVFSDIGAIQSLKRLVSYSTNGTKSALAKRALRLLGEEVPRPILPSVPSWKEAEVQTWLQQIGFSKYCESFREQQVDGDLLLRLTEEELQTDLGMKSGITRKRFFRELTELKTFANYSTCDRSNLADWLGSLDPRFRQYTYGLVSCGLDRSLLHRVSEQQLLEDCGIHLGVHRARILTAAREMLHSPLPCTGGKPSGDTPDVFISYRRNSGSQLASLLKVHLQLHGFSVFIDVEKLEAGKFEDKLIQSVMGARNFVLVLSPGALDKCMQDHDCKDWVHKEIVTALSCGKNIVPIIDGFEWPEPQVLPEDMQAVLTFNGIKWSHEYQEATIEKIIRFLQGRSSRDSSAGSDTSLEGAAPMGPT

SEQ ID NO: 7 - protein, 724 aa, Artificial Sequence
  SYNTHESIZED
MVLTLLLSAYKLCRFFAMSGPRPGAERLAVPGPDGGGGTGPWWAAGGRGPREVSPGAGTEVQDALERALPELQQALSALKQAGGARAVGAGLAEVFQLVEEAWLLPAVGREVAQGLCDAIRLDGGLDLLLRLLQAPELETRVQAARLLEQILVAENRDRVARIGLGVILNLAKEREPVELARSVAGILEHMFMHSEETCQRLVAAGGLDAVLYWCRRTDPALLRHCALALGNCALHGGQAVQRRMVEKRAAEWLFPLAFSKEDELLRLHACLAVAVLATNKEVEREVERSGTLALVEPLVASLDPGRFARCLVDASDTSQGRGPDDLQRLVPLLDSNRLEAQCIGAFYLCAEAAIKSLQGKTKVFSDIGAIQSLKRLVSYSTNGTKSALAKRALRLLGEEVPRPILPSVPSWKEAEVQTWLQQIGFSKYCESFREQQVDGDLLLRLTEEELQTDLGMKSGITRKRFFRELTELKTFANYSTCDRSNLADWLGSLDPRFRQYTYGLVSCGLDRSLLHRVSEQQLLEDCGIHLGVHRARILTAAREMLHSPLPCTGGKPSGDTPDVFISYRRNSGSQLASLLKVHLQLHGFSVFIDVEKLEAGKFEDKLIQSVMGARNFVLVLSPGALDKCMQDHDCKDWVHKEIVTALSCGKNIVPIIDGFEWPEPQVLPEDMQAVLTFNGIKWSHEYQEATIEKIIRFLQGRSSRDSSAGSDTSLEGAAPMGPT

SEQ ID NO: 8 - protein, 724 aa, Artificial Sequence
  SYNTHESIZED
MVLTLLLSAYKLCRFFAMSGPRPGAERLAVPGPDGGGGTGPWWAAGGRGPREVSPGAGTEVQDALERALPELQQALSALKQAGGARAVGAGLAEVFQLVEEAWLLPAVGREVAQGLCDAIRLDGGLDLLLRLLQAPELETRVQAARLLEQILVAENRDRVARIGLGVILNLAKEREPVELARSVAGILEHMFKASEETCQRLVAAGGLDAVLYWCRRTDPALLRHCALALGNCALHGGQAVQRRMVEKRAAEWLFPLAFSKEDELLRLHACLAVAVLATNKEVEREVERSGTLALVEPLVASLDPGRFARCLVDASDTSQGRGPDDLQRLVPLLDSNRLEAQCIGAFYLCAEAAIKSLQGKTKVFSDIGAIQSLKRLVSYSTNGTKSALAKRALRLLGEEVPRPILPSVPSWKEAEVQTWLQQIGFSKYCESFREQQVDGDLLLRLTEEELQTDLGMKSGITRKRFFRELTELKTFANYSTCDRSNLADWLGSLDPRFRQYTYGLVSCGLDRSLLHRVSEQQLLEDCGIHLGVHRARILTAAREMLHSPLPCTGGKPSGDTPDVFISYRRNSGSQLASLLKVHLQLHGFSVFIDVEKLEAGKFEDKLIQSVMGARNFVLVLSPGALDKCMQDHDCKDWVHKEIVTALSCGKNIVPIIDGFEWPEPQVLPEDMQAVLTFNGIKWSHEYQEATIEKIIRFLQGRSSRDSSAGSDTSLEGAAPMGPT

SEQ ID NO: 9 - protein, 724 aa, Artificial Sequence
  SYNTHESIZED
MVLTLLLSAYKLCRFFAMSGPRPGAERLAVPGPDGGGGTGPWWAAGGRGPREVSPGAGTEVQDALERALPELQQALSALKQAGGARAVGAGLAEVFQLVEEAWLLPAVGREVAQGLCDAIRLDGGLDLLLRLLQAPELETRVQAARLLEQILVAENRDRVARIGLGVILNLAKEREPVELARSVAGILEHMFKHSEETCQRLVAAGGLDAVLYWCRRTDPALLRHCALALGNCALHGGQAVQRRMVEKRAAEWLFPLAFSKEDELLRLHACLAVAVLATNKEVEREVERSGTLALVEPLVASLDPGRFARCLVDASDTSQGRGPDDLQRLVPLLDSNRLEAQCIGAFYLCAEAAIKSLQGKTKVFSDIGAIQSLKRLVSYSTNGTKSALAKRALRLLGEEVPRPILPSVPSWKEAEVQTWLQQIGFSKYCESFREQQVDGDLLLRLTEEELQTDLGMKSGITRKRFFRELTELKTFANYSTCDRSNLADWLGSLDPRFRQYTYGLVSCGLDRSLLHRVSEQQLLEDCGIHLGVHRARILTAAREMLHSPLPCTGGKPSGDTPDVFISYRRNSGSQLASLLKVHLQLHGFSVFIDVEKLEAGKFEDKLIQSVMGARNFVLVLSPGALDKCMQDHDCKDWVHKAIVTALSCGKNIVPIIDGFEWPEPQVLPEDMQAVLTFNGIKWSHEYQEATIEKIIRFLQGRSSRDSSAGSDTSLEGAAPMGPT

SEQ ID NO: 10 - protein, 724 aa, Artificial Sequence
  SYNTHESIZED
MVLTLLLSAYKLCRFFAMSGPRPGAERLAVPGPDGGGGTGPWWAAGGRGPREVSPGAGTEVQDALERALPELQQALSALKQAGGARAVGAGLAEVFQLVEEAWLLPAVGREVAQGLCDAIRLDGGLDLLLRLLQAPELETRVQAARLLEQILVAENRDRVARIGLGVILNLAKEREPVELARSVAGILEHMFKHSEETCQRLVAAGGLDAVLYWCRRTDPALLRHCALALGNCALHGGQAVQRRMVEKRAAEWLFPLAFSKEDELLRLHACLAVAVLATNKEVEREVERSGTLALVEPLVASLDPGRFARCLVDASDTSQGRGPDDLQRLVPLLDSNRLEAQCIGAFYLCAEAAIKSLQGKTKVFSDIGAIQSLKRLVSYSTNGTKSALAKRALRLLGEEVPRPILPSVPSWKEAEVQTWLQQIGFSKYCESFREQQVDGDLLLRLTEEELQTDLGMKSGITRKRFFRELTELKTFANYSTCDRSNLADWLGSLDPRFRQYTYGLVSCGLDRSLLHRVSEQQLLEDCGIHLGVHRARILTAAREMLHSPLPCTGGKPSGDTPDVFISYRRNSGSQLASLLKVHLQLHGFSVFIDVEKLEAGKFEDKLIQSVMGARNFVLVLSPGALDKCMQDHDCKDWVHKEIVTALSCGKNIVPIIDGFEWPEPQVLPEDMQAVLTFNGIKWSAEYQEATIEKIIRFLQGRSSRDSSAGSDTSLEGAAPMGPT

SEQ ID NO: 11 - protein, 724 aa, Artificial Sequence
  SYNTHESIZED
MVLTLLLSAYKLCRFFAMSGPRPGAERLAVPGPDGGGGTGPWWAAGGRGPREVSPGAGTEVQDALERALPELQQALSALKQAGGARAVGAGLAEVFQLVEEAWLLPAVGREVAQGLCDAIRLDGGLDLLLRLLQAPELETRVQAARLLEQILVAENRDRVARIGLGVILNLAKEREPVELARSVAGILEHMFRHSEETCQRLVAAGGLDAVLYWCRRTDPALLRHCALALGNCALHGGQAVQRRMVEKRAAEWLFPLAFSKEDELLRLHACLAVAVLATNKEVEREVERSGTLALVEPLVASLDPGRFARCLVDASDTSQGRGPDDLQRLVPLLDSNRLEAQCIGAFYLCAEAAIKSLQGKTKVFSDIGAIQSLKRLVSYSTNGTKSALAKRALRLLGEEVPRPILPSVPSWKEAEVQTWLQQIGFSKYCESFREQQVDGDLLLRLTEEELQTDLGMKSGITRKRFFRELTELKTFANYSTCDRSNLADWLGSLDPRFRQYTYGLVSCGLDRSLLHRVSEQQLLEDCGIHLGVHRARILTAAREMLHSPLPCTGGKPSGDTPDVFISYRRNSGSQLASLLKVHLQLHGFSVFIDVEKLEAGKFEDKLIQSVMGARNFVLVLSPGALDKCMQDHDCKDWVHKAIVTALSCGKNIVPIIDGFEWPEPQVLPEDMQAVLTFNGIKWSHEYQEATIEKIIRFLQGRSSRDSSAGSDTSLEGAAPMGPT

SEQ ID NO: 12 - protein, 724 aa, Artificial Sequence
  SYNTHESIZED
MVLTLLLSAYKLCRFFAMSGPRPGAERLAVPGPDGGGGTGPWWAAGGRGPREVSPGAGTEVQDALERALPELQQALSALKQAGGARAVGAGLAEVFQLVEEAWLLPAVGREVAQGLCDAIRLDGGLDLLLRLLQAPELETRVQAARLLEQILVAENRDRVARIGLGVILNLAKEREPVELARSVAGILEHMFKHSEETCQRLVAAGGLDAVLYWCRRTDPALLRHCALALGNCALHGGQAVQRRMVEKRAAEWLFPLAFSKEDELLRLHACLAVAVLATNKEVEREVERSGTLALVEPLVASLDPGRFARCLVDASDTSQGRGPDDLQRLVPLLDSNRLEAQCIGAFYLCAEAAIKSLQGKTKVFSDIGAIQSLKRLVSYSTNGTKSALAKRALRLLGEEVPRPILPSVPSWKEAEVQTWLQQIGFSKYCESFREQQVDGDLLLRLTEEELQTDLGMKSGITRKRFFRELTELKTFANYSTCDRSNLADWLGSLDPRFRQYTYGLVSCGLDRSLLHRVSEQQLLEDCGIHLGVHRARILTAAREMLHSPLPCTGGKPSGDTPDVFISYRRNSGSQLASLLKVHLQLHGFSVFIDVEKLEAGKFEDKLIQSVMGARNFVLVLSPGALDKCMQDHDCKDWVHKAIVTALSCGKNIVPIIDGFEWPEPQVLPEDMQAVLTFNGIKWSAEYQEATIEKIIRFLQGRSSRDSSAGSDTSLEGAAPMGPT

SEQ ID NO: 13 - protein, 724 aa, Artificial Sequence
  SYNTHESIZED
MVLTLLLSAYKLCRFFAMSGPRPGAERLAVPGPDGGGGTGPWWAAGGRGPREVSPGAGTEVQDALERALPELQQALSALKQAGGARAVGAGLAEVFQLVEEAWLLPAVGREVAQGLCDAIRLDGGLDLLLRLLQAPELETRVQAARLLEQILVAENRDRVARIGLGVILNLAKEREPVELARSVAGILEHMFRHSEETCQRLVAAGGLDAVLYWCRRTDPALLRHCALALGNCALHGGQAVQRRMVEKRAAEWLFPLAFSKEDELLRLHACLAVAVLATNKEVEREVERSGTLALVEPLVASLDPGRFARCLVDASDTSQGRGPDDLQRLVPLLDSNRLEAQCIGAFYLCAEAAIKSLQGKTKVFSDIGAIQSLKRLVSYSTNGTKSALAKRALRLLGEEVPRPILPSVPSWKEAEVQTWLQQIGFSKYCESFREQQVDGDLLLRLTEEELQTDLGMKSGITRKRFFRELTELKTFANYSTCDRSNLADWLGSLDPRFRQYTYGLVSCGLDRSLLHRVSEQQLLEDCGIHLGVHRARILTAAREMLHSPLPCTGGKPSGDTPDVFISYRRNSGSQLASLLKVHLQLHGFSVFIDVEKLEAGKFEDKLIQSVMGARNFVLVLSPGALDKCMQDHDCKDWVHKEIVTALSCGKNIVPIIDGFEWPEPQVLPEDMQAVLTFNGIKWSAEYQEATIEKIIRFLQGRSSRDSSAGSDTSLEGAAPMGPT

SEQ ID NO: 14 - protein, 724 aa, Artificial Sequence
  SYNTHESIZED
MVLTLLLSAYKLCRFFAMSGPRPGAERLAVPGPDGGGGTGPWWAAGGRGPREVSPGAGTEVQDALERALPELQQALSALKQAGGARAVGAGLAEVFQLVEEAWLLPAVGREVAQGLCDAIRLDGGLDLLLRLLQAPELETRVQAARLLEQILVAENRDRVARIGLGVILNLAKEREPVELARSVAGILEHMFRHSEETCQRLVAAGGLDAVLYWCRRTDPALLRHCALALGNCALHGGQAVQRRMVEKRAAEWLFPLAFSKEDELLRLHACLAVAVLATNKEVEREVERSGTLALVEPLVASLDPGRFARCLVDASDTSQGRGPDDLQRLVPLLDSNRLEAQCIGAFYLCAEAAIKSLQGKTKVFSDIGAIQSLKRLVSYSTNGTKSALAKRALRLLGEEVPRPILPSVPSWKEAEVQTWLQQIGFSKYCESFREQQVDGDLLLRLTEEELQTDLGMKSGITRKRFFRELTELKTFANYSTCDRSNLADWLGSLDPRFRQYTYGLVSCGLDRSLLHRVSEQQLLEDCGIHLGVHRARILTAAREMLHSPLPCTGGKPSGDTPDVFISYRRNSGSQLASLLKVHLQLHGFSVFIDVEKLEAGKFEDKLIQSVMGARNFVLVLSPGALDKCMQDHDCKDWVHKAIVTALSCGKNIVPIIDGFEWPEPQVLPEDMQAVLTFNGIKWSAEYQEATIEKIIRFLQGRSSRDSSAGSDTSLEGAAPMGPT

SEQ ID NO: 15 - DNA, 2172 bp, Artificial Sequence
  SYNTHESIZED
atggtcctgacgctgcttctctccgcctacaagctgtgtcgcttcttcgccatgtcgggcccacggccgggcgccgagcggctggcggtgcctgggccagatgggggcggtggcacgggcccatggtgggctgcgggtggccgcgggccccgcgaagtgtcgccgggggcaggcaccgaggtgcaggacgccctggagcgcgcgctgccggagctgcagcaggccttgtccgcgctgaagcaggcgggcggcgcgcgggccgtgggcgccggcctggccgaggtcttccaactggtggaggaggcctggctgctgccggccgtgggccgcgaggtagcccagggtctgtgcgacgccatccgcctcgatggcggcctcgacctgctgttgcggctgctgcaggcgccggagttggagacgcgtgtgcaggccgcgcgcctgctggagcagatcctggtggctgagaaccgagaccgcgtggcgcgcattgggctgggcgtgatcctgaacctggcgaaggaacgcgaacccgtagagctggcgcggagcgtggcaggcatcttggagcacatgttccggcattcggaggagacatgccagaggctggtggcggccggcggcctggacgcggtgctgtattggtgccgccgcacggaccccgcgctgctgcgccactgcgcgctggcgctgggcaactgcgcgctgcacgggggccaggcggtgcagcgacgcatggtagagaagcgcgcagccgagtggctcttcccgctcgccttctccaaggaggacgagctgcttcggctgcacgcctgcctcgcagtagcggtgttggcgactaacaaggaggtggagcgcgaggtggagcgctcgggcacgctggcgctcgtggagccgcttgtggcctcgctggaccctggccgcttcgcccgctgtctggtggacgccagcgacacaagccagggccgcgggcccgacgacctgcagcgcctcgtgccgttgctcgactctaaccgcttggaggcgcagtgcatcggggctttctacctctgcgccgaggctgccatcaagagcctgcaaggcaagaccaaggtgttcagcgacatcggcgccatccagagcctgaaacgcctggtttcctactctaccaatggcactaagtcggcgctggccaagcgcgcgctgcgcctgctgggcgaggaggtgccacggcccatcctgccctccgtgcccagctggaaggaggccgaggttcagacgtggctgcagcagatcggtttctccaagtactgcgagagcttccgggagcagcaggtggatggcgacctgcttctgcggctcacggaggaggaactccagaccgacctgggcatgaaatcgggcatcacccgcaagaggttctttagggagctcacggagctcaagaccttcgccaactattctacgtgcgaccgcagcaacctggcggactggctgggcagcctggacccgcgcttccgccagtacacctacggcctggtcagctgcggcctggaccgctccctgctgcaccgcgtgtctgagcagcagctgctggaagactgcggcatccacctgggcgtgcaccgcgcccgcatcctcacggcggccagagaaatgctacactccccgctgccctgtactggtggcaaacccagtggggacactccagatgtcttcatcagctaccgccggaactcaggttcccagctggccagtctcctgaaggtgcacctgcagctgcatggcttcagtgtcttcattgatgtggagaagctggaagcaggcaagttcgaggacaaactcatccagagtgtcatgggtgcccgcaactttgtgttggtgctatcacctggagcactggacaagtgcatgcaagaccatgactgcaaggattgggtgcataaggagattgtgactgctttaagctgcggcaagaacattgtgcccatcattgatggcttcgagtggcctgagccccaggtcctgcctgaggacatgcaggctgtgcttactttcaacggtatcaagtggtccgccgaataccaggaggccaccattgagaagatcatccgcttcctgcagggccgctcctcccgggactcatctgcaggctctgacaccagtttggagggtgctgcacccatgggtccaacc